European Patent Application EP 4 276 113 A1, published November 15, 2023. Title: ANTIBODY SPECIFICALLY BINDING TO CD47 AND ANTIGEN-BINDING FRAGMENT THEREOF. Applicant: BEIJING HANMI PHARMACEUTICAL CO., LTD. The sequence listing filed with the application follows.

SEQUENCE LISTING (37 sequences)

SEQ ID NO: 1 - protein, 11 aa, Artificial
  LCDR1
KASQNVRTSIA

SEQ ID NO: 2 - protein, 7 aa, Artificial
  LCDR2
LASNRHT

SEQ ID NO: 3 - protein, 9 aa, Artificial
  LCDR3
LQHWNYPFT

SEQ ID NO: 4 - protein, 10 aa, Artificial
  HCDR1
GFNIEDIYMH

SEQ ID NO: 5 - protein, 17 aa, Artificial
  HCDR2
RIDPANDNTKYGPKLQG

SEQ ID NO: 6 - protein, 17 aa, Artificial
  HCDR2
RIDPANDNTKYGPKFQG

SEQ ID NO: 7 - protein, 9 aa, Artificial
  HCDR3
RIPTDIMDY

SEQ ID NO: 8 - protein, 9 aa, Artificial
  HCDR3
RITTDVMDY

SEQ ID NO: 9 - protein, 107 aa, Artificial
  Light chain variable region
DIVMTQSQKFMSTSVGDRVSITCKASQNVRTSIAWYQQKSGQSPKTLIYLASNRHTGVPDRFTGSGSGTDFTLTISNVQSEDLADYFCLQHWNYPFTFGSGTKLEIK

SEQ ID NO: 10 - protein, 107 aa, Artificial
  Light chain variable region
DIVMTQSQKFMSTSVGDRVSITCKASQNVRTSIAWYQQKPGQSPKTLIYLASNRHTGVPDRFTGSGSGTDFTLTISNVQSEDLADYFCLQHWNYPFTFGSGTKLEIK

SEQ ID NO: 11 - protein, 118 aa, Artificial
  Heavy chain variable region
EVQLQQSGAELVKPGASVKLSCTASGFNIEDIYMHWVKQRPEQGLEWIGRIDPANDNTKYGPKLQGRATITADTSSNTAYLQLSGLTSEDTGVYYCVRRIPTDIMDYWGPGTSVTVSS

SEQ ID NO: 12 - protein, 118 aa, Artificial
  Heavy chain variable region
EVQLQQSGAELVKPGASVKLSCTASGFNIEDIYMHWVKQRPEQGLEWIGRIDPANDNTKYGPKFQGRATMTADTSSNTAYLQLSGLTSEDTGVYYCVRRITTDVMDYWGQGTSVTVSS

SEQ ID NO: 13 - protein, 107 aa, Artificial [sequence omitted]

SEQ ID NO: 14 - protein, 330 aa, Artificial [sequence omitted]

SEQ ID NO: 15 - protein, 330 aa, Artificial
  Heavy chain constant region
ASTKGPSVFPLAPSSKSTSGGTAALGCLVKDYFPEPVTVSWNSGALTSGVHTFPAVLQSSGLYSLSSVVTVPSSSLGTQTYICNVNHKPSNTKVDKKVEPKSCDKTHTCPPCPAPELLGGPSVFLFPPKPKDTLMISRTPEVTCVVVDVSHEDPEVKFNWYVDGVEVHNAKTKPREEQYASTYRVVSVLTVLHQDWLNGKEYKCKVSNKALPAPIEKTISKAKGQPREPQVYTLPPSRDELTKNQVSLTCLVKGFYPSDIAVEWESNGQPENNYKTTPPVLDSDGSFFLYSKLTVDKSRWQQGNVFSCSVMHEALHNHYTQKSLSLSPGK

SEQ ID NO: 16 - protein, 327 aa, Artificial
  Heavy chain constant region
ASTKGPSVFPLAPCSRSTSESTAALGCLVKDYFPEPVTVSWNSGALTSGVHTFPAVLQSSGLYSLSSVVTVPSSSLGTKTYTCNVDHKPSNTKVDKRVESKYGPPCPPCPAPEFLGGPSVFLFPPKPKDTLMISRTPEVTCVVVDVSQEDPEVQFNWYVDGVEVHNAKTKPREEQFNSTYRVVSVLTVLHQDWLNGKEYKCKVSNKGLPSSIEKTISKAKGQPREPQVYTLPPSQEEMTKNQVSLTCLVKGFYPSDIAVEWESNGQPENNYKTTPPVLDSDGSFFLYSRLTVDKSRWQEGNVFSCSVMHEALHNHYTQKSLSLSLGK

SEQ ID NO: 17 - protein, 23 aa, Artificial
  FR-L1
DIQMTQSPSSLSASVGDRVTITC

SEQ ID NO: 18 - protein, 15 aa, Artificial
  FR-L2
WYQQKPGKAPKRLIY

SEQ ID NO: 19 - protein, 32 aa, Artificial
  FR-L3
GVPSRFSGSGSGTEFTLTISNLQPEDFATYYC

SEQ ID NO: 20 - protein, 10 aa, Artificial
  FR-L4
FGQGTKLEIK

SEQ ID NO: 21 - protein, 25 aa, Artificial [sequence omitted]

SEQ ID NO: 22 - protein, 14 aa, Artificial
  FR-H2
WVRQAPGQGLEWMG

SEQ ID NO: 23 - protein, 32 aa, Artificial
  FR-H3
RVTITADESTSTAYMELSSLRSEDTAVYYCAR

SEQ ID NO: 24 - protein, 11 aa, Artificial
  FR-H4
WGQGTTVTVSS

SEQ ID NO: 25 - protein, 107 aa, Artificial
  Light chain variable region
DIQMTQSPSSLSASVGDRVTITCKASQNVRTSIAWYQQKPGKAPKRLIYLASNRHTGVPSRFSGSGSGTEFTLTISNLQPEDFATYYCLQHWNYPFTFGQGTKLEIK

SEQ ID NO: 26 - protein, 107 aa, Artificial
  Light chain variable region
DIQMTQSPSSLSASVGDRVTITCKASQNVRTSIAWYQQKPGKAPKTLIYLASNRHTGVPSRFSGSGSGTEFTLTISNLQPEDFATYYCLQHWNYPFTFGQGTKLEIK

SEQ ID NO: 27 - protein, 107 aa, Artificial
  Light chain variable region
DIQMTQSPSSLSASVGDRVTITCKASQNVRTSIAWYQQKPGKAPKTLIYLASNRHTGVPSRFSGSGSGTEFTLTISNLQPEDFATYFCLQHWNYPFTFGQGTKLEIK

SEQ ID NO: 28 - protein, 118 aa, Artificial
  Heavy chain variable region
QVQLVQSGAEVKKPGSSVKVSCKASGFNIEDIYMHWVRQAPGQGLEWMGRIDPANDNTKYGPKLQGRVTITADESTSTAYMELSSLRSEDTAVYYCARRIPTDIMDYWGQGTTVTVSS

SEQ ID NO: 29 - protein, 118 aa, Artificial
  Heavy chain variable region
QVQLVQSGAEVKKPGSSVKVSCKASGFNIEDIYMHWVRQAPGQGLEWMGRIDPANDNTKYGPKLQGRVTITADESTSTAYMELSSLRSEDTAVYYCVRRIPTDIMDYWGQGTTVTVSS

SEQ ID NO: 30 - protein, 118 aa, Artificial
  Heavy chain variable region
QVQLVQSGAEVKKPGSSVKVSCKASGFNIEDIYMHWVRQAPGQGLEWMGRIDPANDNTKYGPKLQGRVTITADTSTSTAYMELSSLRSEDTAVYYCARRIPTDIMDYWGQGTTVTVSS

SEQ ID NO: 31 - protein, 118 aa, Artificial
  Heavy chain variable region
QVQLVQSGAEVKKPGSSVKVSCKASGFNIEDIYMHWVRQAPGQGLEWMGRIDPANDNTKYGPKLQGRVTITADESTNTAYMELSSLRSEDTAVYYCARRIPTDIMDYWGQGTTVTVSS

SEQ ID NO: 32 - protein, 118 aa, Artificial
  Heavy chain variable region
QVQLVQSGAEVKKPGSSVKVSCKASGFNIEDIYMHWVRQAPGQGLEWMGRIDPANDNTKYGPKLQGRVTITADTSTSTAYMELSSLRSEDTAVYYCVRRIPTDIMDYWGQGTTVTVSS

SEQ ID NO: 33 - protein, 118 aa, Artificial
  Heavy chain variable region
QVQLVQSGAEVKKPGSSVKVSCKASGFNIEDIYMHWVRQAPGQGLEWMGRIDPANDNTKYGPKLQGRVTITADTSTNTAYMELSSLRSEDTAVYYCVRRIPTDIMDYWGQGTTVTVSS

SEQ ID NO: 34 - protein, 95 aa, Artificial
  IGKV1-17*02
DIQMTQSPSSLSASVGDRVTITCRASQGIRNDLGWYQQKPGKAPKRLIYAASSLQSGVPSRFSGSGSGTEFTLTISNLQPEDFATYYCLQHNSYP

SEQ ID NO: 35 - protein, 98 aa, Artificial
  IGHV1-69*01
QVQLVQSGAEVKKPGSSVKVSCKASGGTFSSYAISWVRQAPGQGLEWMGGIIPIFGTANYAQKFQGRVTITADESTSTAYMELSSLRSEDTAVYYCAR

SEQ ID NO: 36 - DNA, 47 bp, Artificial
  Primer VHGSP
gattacgccaagcttgccagtggatagacaagcttgggtgtcgtttt

SEQ ID NO: 37 - DNA, 42 bp, Artificial
  Primer VLGSP
gattacgccaagcttgatggatccagttggtgcagcatcagc